European Patent Application EP 4 729 126 A1, published April 22, 2026. Title: NK CELL-DERIVED EXTRACELLULAR VESICLES ARMED WITH MODIFIED MONOCLONAL ANTIBODIES TO TARGET CANCER CELLS, AND USE THEREOF. Applicant: Universite de Montpellier. Application EP N/A. The sequence listing filed with the application follows.

SEQUENCE LISTING (8 sequences)

SEQ ID NO: 1 - protein, 110 aa, synthetic construct
APELLGGPSVFLFPPKPKDTLMISRTPEVTCVVVDVSHEDPEVKFNWYVDGVEVHNAKTKPREEQYNSTYRVVSVLTVLHQDWLNGKEYKCKVSNKALPAPIEKTISKAK

SEQ ID NO: 2 - protein, 110 aa, synthetic construct
APELLGGPDVFLFPPKPKDTLMISRTPEVTCVVVDVSHEDPEVKFNWYVDGVEVHNAKTKPREEQYNSTYRVVSVLTVLHQDWLNGKEYKCKVSNKALPAPIEKTISKAK

SEQ ID NO: 3 - protein, 110 aa, synthetic construct
APELLGGPSVFLFPPKPKDTLMISRTPEVTCVVVDVSHEDPEVKFNWYVDGVEVHNAKTKPREEQYNSTYRVVSVLTVLHQDWLNGKEYKCKVSNKALPAPEEKTISKAK

SEQ ID NO: 4 - protein, 110 aa, synthetic construct
APELLGGPSVFLFPPKPKDTLMISRTPEVTCVVVDVSFEDPEVKFNWYVDGVEVHNAKTKPREEQYNSTYRVVSVLTVLHQDWLNGKEYKCKVSNKALPAPIEKTISKAK

SEQ ID NO: 5 - protein, 110 aa, synthetic construct
APELLGGPSVFLFPPKPKDTLMISRTPEVTCVVVDVSHEDPEVKFNWYVDGVEVHNAKTKPREEQYNSTYRVVSVLTVLHQDWLNGKEYKCKVTNKALPAPIEKTISKAK

SEQ ID NO: 6 - protein, 110 aa, synthetic construct
APELLAGPSVFLFPPKPKDTLMISRTPEVTCVVVDVSHEDPEVKFNWYVDGVEVHNAKTKPREEQYNSTYRVVSVLTVLHQDWLNGKEYKCKVSNKALPAPIEKTISKAK

SEQ ID NO: 7 - protein, 110 aa, synthetic construct
APELLGGPDVFLFPPKPKDTLMISRTPEVTCVVVDVSHEDPEVKFNWYVDGVEVHNAKTKPREEQYNSTYRVVSVLTVLHQDWLNGKEYKCKVSNKALPLPIEKTISKAK

SEQ ID NO: 8 - protein, 110 aa, synthetic construct
APELLGGPDVFLFPPKPKDTLMISRTPEVTCVVVDVSFEDPEVKFNWYVDGVEVHNAKTKPREEQYNSTYRVVSVLTVLHQDWLNGKEYKCKVTNKALPAPEEKTISKAK